European Patent Application EP 4 458 966 A1, published November 6, 2024. Title: METHODE DE DETECTION DE MICROALGUES. Applicant: SUEZ INTERNATIONAL. Application EP. The sequence listing filed with the application follows.

SEQUENCE LISTING (14 sequences)

SEQ ID NO: 1 - DNA, 22 bp, synthetic construct
  source 1..22: mol_type = other DNA; note = amorce anti-sens Ostreopsis
ccargaryatgcctacattcaa

SEQ ID NO: 2 - DNA, 20 bp, synthetic construct
  source 1..20: mol_type = other DNA; note = amorce sens siamensis
tgttaccattgctgagtttg

SEQ ID NO: 3 - DNA, 20 bp, synthetic construct
  source 1..20: mol_type = other DNA; note = amorce sens ovata
caatgctcatgtcaatgatg

SEQ ID NO: 4 - DNA, 22 bp, synthetic construct
  source 1..22: mol_type = other DNA; note = amorce sens Ostreopsis
aaaacgatatgaagagtgcagc

SEQ ID NO: 5 - DNA, 22 bp, synthetic construct
  source 1..22: mol_type = other DNA; note = amorce anti-sens Ostreopsis
ccaggagtatgcctacattcaa

SEQ ID NO: 6 - DNA, 22 bp, synthetic construct
  source 1..22: mol_type = other DNA; note = amorce anti-sens ovata
ccaggagcatgcctacattcaa

SEQ ID NO: 7 - DNA, 22 bp, synthetic construct
  source 1..22: mol_type = other DNA; note = amorce anti-sens ovata
ccaggaatatgcctacattcaa

SEQ ID NO: 8 - DNA, 22 bp, synthetic construct
  source 1..22: mol_type = other DNA; note = amorce anti-sens ovata
ccaggaacatgcctacattcaa

SEQ ID NO: 9 - DNA, 22 bp, synthetic construct
  source 1..22: mol_type = other DNA; note = amorce anti-sens ovata
ccaagagtatgcctacattcaa

SEQ ID NO: 10 - DNA, 22 bp, synthetic construct
  source 1..22: mol_type = other DNA; note = amorce anti-sens ovata
ccaagagcatgcctacattcaa

SEQ ID NO: 11 - DNA, 22 bp, synthetic construct
  source 1..22: mol_type = other DNA; note = amorce anti-sens ovata
ccaagaatatgcctacattcaa

SEQ ID NO: 12 - DNA, 22 bp, synthetic construct
  source 1..22: mol_type = other DNA; note = amorce anti-sens ovata
ccaagaacatgcctacattcaa

SEQ ID NO: 13 - DNA, 323 bp, synthetic construct
  source 1..323: mol_type = other DNA; note = sequence consus Ostreopsis cf. siamensis
ttcacaatgaatttttccgtaggtgaacctgcggaaggatcatttgtgaatgttaccattgctgagtttgtgtgtatcttgcacatgcatgtaaacacatatgcttcactataagtttgcatatctgatcagtgtgctgtccttgacttcattttagttgcagcaatgaatgcatcaattcaaaacgatatgaagagtgcagccaattgcattaattattgcaaattgcagaattccgtgagtcatttttcttgaatgtaggcatactcctgggccattcctgagagcattatttgttcagtgttcattgctatatatatgat

SEQ ID NO: 14 - DNA, 311 bp, synthetic construct
  source 1..311: mol_type = other DNA; note = sequence consensus Ostreopsis cf. ovata
gatggtaacagggttcgccgtaggtgaacctgcagaaggatcatttgtgaacaatgctcatgtcaatgatgcttggtggcatgcaccttgttagttgtagcatgacagcttgatacttatctaaacgctttcatcaactgtcttctgacagcaatgaatgcatcaattcaaaacaatatgaagagtgcagccaaatgcagtaatcattgcaaattgcagaattccgtgagtcatttttcttgaatgtaggcatgttcttgggccacccctaaggacatcatttactcagtgcatctttgttaatggtgtgc